European Patent Application EP 4 206 229 A1, published July 5, 2023. Title: A BINDING MOLECULE ABLE TO NEUTRALIZE PROX1 PROTEIN. Applicant: Korea Advanced Institute of Science and Technology. Application EP. The sequence listing filed with the application follows.

SEQUENCE LISTING (15 sequences)

SEQ ID NO: 1 - protein, 282 aa, synthetic construct
  REGION 1..282: note = anti-PROX1-single chain Fv-His
LTQPSSVSANLGETVEITCSGGSGSYGWYQQKSPGSAPVTLIYDNANRPSNIPSRFSGSKSGSTGTLTITGVRAEDEAVYYCGNVDSSTYVGMFGAGTTLTVLGQSSRSSGGGGSSGGGGSAVTLDESGGGLQTPGGGLSLVCKASGFTFSSYAMNWVRQAPGKGLEWVAAIDDDGSYTGYGSAVKGRATISRDNGQSTVRLQLNNLRAEDTAIYYCAKAAGSGYCYRGANSSYTCGTYNAGDIDAWGHGTEVIVSSTSGQAGQHHHHHHGAYPYDVPDYAS

SEQ ID NO: 2 - DNA, 1224 bp, synthetic construct
  misc_feature 1..1224: note = anti-PROX1-single chain Fv-His
  source 1..1224: mol_type = other DNA
aacctgagattaaatgagaagacagctatcgcgattgcagtggcactggctggtttcgctaccgtggcccaggcggccctgactcagccgtcctcggtgtcagcaaacctaggagaaaccgtcgagatcacctgctccgggggtagtggcagctatggctggtatcagcagaagtcacctggcagtgcccctgtcactctgatctatgacaacgccaacagaccctcgaacatcccttcacgattctccggttccaaatccggctccacgggcacattaaccatcactggggtccgagccgaggatgaggctgtctattactgtgggaatgtagacagcagcacttatgttggtatgtttggggccgggacaaccctgaccgtcctaggtcagtcctctagatcttccggcggtggtggcagctccggtggtggcggttccgccgtgacgttggacgagtccgggggcggcctccagacgcccggaggagggctcagcctcgtctgcaaggcctccgggttcaccttcagcagttatgccatgaactgggtgcgacaggcgcccggcaaggggctggagtgggtcgctgctattgatgatgatggtagttacacaggctacgggtcggcggtgaagggccgtgccaccatctcgagggacaacgggcagagcacagtgaggctgcagctgaacaacctcagggctgaggacaccgccatctactactgcgccaaagctgctggtagtggttactgttatcgtggtgctaatagtagttatacttgtggtacttataacgctggtgacatcgacgcatggggccacgggaccgaagtcatcgtctcctccactagtggccaggccggccagcaccatcaccatcaccatggcgcatacccgtacgacgttccggactacgcttcttaggagggtggtggctctgagggtggcggttctgagggtggcggctctgagggaggcggttccggtggtggctctggttccggtgattttgattatgaaaagatggcaaacgctaataagggggctatgaccgaaaatgccgatgaaaacgtgctacagtctgacgctaaaggcaaacttgattctgtcgctactgattacggtgctgctatcgatggtttcattggtgacgtttccggccttgctaatggtaatggtgctactggggattttgctggctctaattcccaaatggctcag

SEQ ID NO: 3 - protein, 103 aa, synthetic construct
  REGION 1..103: note = anti-PROX1-single chain Fv-His light chain
LTQPSSVSANLGETVEITCSGGSGSYGWYQQKSPGSAPVTLIYDNANRPSNIPSRFSGSKSGSTGTLTITGVRAEDEAVYYCGNVDSSTYVGMFGAGTTLTVL

SEQ ID NO: 4 - protein, 138 aa, synthetic construct
  REGION 1..138: note = anti-PROX1-single chain Fv-His heavy chain
AVTLDESGGGLQTPGGGLSLVCKASGFTFSSYAMNWVRQAPGKGLEWVAAIDDDGSYTGYGSAVKGRATISRDNGQSTVRLQLNNLRAEDTAIYYCAKAAGSGYCYRGANSSYTCGTYNAGDIDAWGHGTEVIVSSTS

SEQ ID NO: 5 - protein, 18 aa, synthetic construct
  REGION 1..18: note = anti-PROX1-single chain Fv-His linker
GQSSRSSGGGGSSGGGGS

SEQ ID NO: 6 - protein, 7 aa, synthetic construct
  REGION 1..7: note = anti-PROX1-single chain Fv-His CDR1
GGSGSYG

SEQ ID NO: 7 - protein, 4 aa, synthetic construct
  REGION 1..4: note = anti-PROX1-single chain Fv-His CDR2
DNAN

SEQ ID NO: 8 - protein, 8 aa, synthetic construct
  REGION 1..8: note = anti-PROX1-single chain Fv-His CDR3
GNVDSSTY

SEQ ID NO: 9 - protein, 5 aa, synthetic construct
  REGION 1..5: note = anti-PROX1-single chain Fv-His CDR4
SYAMN

SEQ ID NO: 10 - protein, 10 aa, synthetic construct
  REGION 1..10: note = anti-PROX1-single chain Fv-His CDR5
IDDDGSYTGY

SEQ ID NO: 11 - protein, 28 aa, synthetic construct
  REGION 1..28: note = anti-PROX1-single chain Fv-His CDR6
KAAGSGYCYRGANSSYTCGTYNAGDIDA

SEQ ID NO: 12 - protein, 515 aa, synthetic construct
  REGION 1..515: note = anti-PROX1-scFv-hFc
METDTLLLWVLLLLAAQPALTQPSSVSANLGETVEITCSGGSGSYGWYQQKSPGSAPVTLIYDNANRPSNIPSRFSGSKSGSTGTLTITGVRAEDEAVYYCGNVDSSTYVGMFGAGTTLTVLGQSSRSSGGGGSSGGGGSAVTLDESGGGLQTPGGGLSLVCKASGFTFSSYAMNWVRQAPGKGLEWVAAIDDDGSYTGYGSAVKGRATISRDNGQSTVRLQLNNLRAEDTAIYYCAKAAGSGYCYRGANSSYTCGTYNAGDIDAWGHGTEVIVSSTSGPGGPEPKSSDKTHTCPPCPAPELLGGPSVFLFPPKPKDTLMISRTPEVTCVVVDVSHEDPEVKFNWYVDGVEVHNAKTKPREEQYNSTYRVVSVLTVLHQDWLNGKEYKCKVSNKALPAPIEKTISKAKGQPREPQVYTLPPSRDELTKNQVSLTCLVKGFYPSDIAVEWESNGQPENNYKTTPPVLDSDGSFFLYSKLTVDKSRWQQGNVFSCSVMHEALHNHYTQKSLSLSPGK

SEQ ID NO: 13 - DNA, 1548 bp, synthetic construct
  misc_feature 1..1548: note = anti-PROX1-scFv-hFc
  source 1..1548: mol_type = other DNA
atggagacagacacactcctgctatgggtactgctgctcttagcggcccagccggccctgactcagccgtcctcggtgtcagcaaacctaggagaaaccgtcgagatcacctgctccgggggtagtggcagctatggctggtatcagcagaagtcacctggcagtgcccctgtcactctgatctatgacaacgccaacagaccctcgaacatcccttcacgattctccggttccaaatccggctccacgggcacattaaccatcactggggtccgagccgaggatgaggctgtctattactgtgggaatgtagacagcagcacttatgttggtatgtttggggccgggacaaccctgaccgtcctaggtcagtcctctagatcttccggcggtggtggcagctccggtggtggcggttccgccgtgacgttggacgagtccgggggcggcctccagacgcccggaggagggctcagcctcgtctgcaaggcctccgggttcaccttcagcagttatgccatgaactgggtgcgacaggcgcccggcaaggggctggagtgggtcgctgctattgatgatgatggtagttacacaggctacgggtcggcggtgaagggccgtgccaccatctcgagggacaacgggcagagcacagtgaggctgcagctgaacaacctcagggctgaggacaccgccatctactactgcgccaaagctgctggtagtggttactgttatcgtggtgctaatagtagttatacttgtggtacttataacgctggtgacatcgacgcatggggccacgggaccgaagtcatcgtctcctccactagtggcccgggaggccccgagcccaaatcttctgacaaaactcacacatgcccaccgtgcccagcacctgaactcctggggggaccgtcagtcttcctcttccccccaaaacccaaggacaccctcatgatctcccggacccctgaggtcacatgcgtggtggtggacgtgagccacgaagaccctgaggtcaagttcaactggtacgtggacggcgtggaggtgcataatgccaagacaaagccgcgggaggagcagtacaacagcacgtaccgtgtggtcagcgtcctcaccgtcctgcaccaggactggctgaatggcaaggagtacaagtgcaaggtgtccaacaaagccctcccagcccccatcgagaaaaccatctccaaagccaaagggcagccccgagaaccacaggtgtacaccctgcccccatcccgggatgagctgaccaagaaccaggtcagcctgacctgcctggtcaaaggcttctatcccagcgacatcgccgtggagtgggagagcaatgggcagccggagaacaactacaagaccacgcctcccgtgctggactccgacggctccttcttcctctatagcaagctcaccgtggacaagagcaggtggcagcaggggaacgtcttctcatgctccgtgatgcatgaggctctgcacaaccactacacgcagaagagcctctccctgtctccgggtaaatga

SEQ ID NO: 14 - protein, 294 aa, synthetic construct
  REGION 1..294: note = AAV2/2-IL2'SP-anti-PROX1-scFv-Flag
MYRMQLLSCIALSLALVTNSMLTQPSSVSANLGETVEITCSGGSGSYGWYQQKSPGSAPVTLIYDNANRPSNIPSRFSGSKSGSTGTLTITGVRAEDEAVYYCGNVDSSTYVGMFGAGTTLTVLGQSSRSSGGGGSSGGGGSAVTLDESGGGLQTPGGGLSLVCKASGFTFSSYAMNWVRQAPGKGLEWVAAIDDDGSYTGYGSAVKGRATISRDNGQSTVRLQLNNLRAEDTAIYYCAKAAGSGYCYRGANSSYTCGTYNAGDIDAWGHGTEVIVSSTSGQAGQMDYKDDDDK

SEQ ID NO: 15 - DNA, 888 bp, synthetic construct
  misc_feature 1..888: note = AAV2/2-IL2'SP-anti-PROX1-scFv-Flag
  source 1..888: mol_type = other DNA
atgtacagaatgcaactcctgtcttgtattgcactaagtctcgcacttgtcacaaacagtatgctgactcagccgtcctcggtgtcagcaaacctaggagaaaccgtcgagatcacctgctccgggggtagtggcagctatggctggtatcagcagaagtcacctggcagtgcccctgtcactctgatctatgacaacgccaacagaccctcgaacatcccttcacgattctccggttccaaatccggctccacgggcacattaaccatcactggggtccgagccgaggatgaggctgtctattactgtgggaatgtagacagcagcacttatgttggtatgtttggggccgggacaaccctgaccgtcctaggtcagtcctctagatcttccggcggtggtggcagctccggtggtggcggttccgccgtgacgttggacgagtccgggggcggcctccagacgcccggaggagggctcagcctcgtctgcaaggcctccgggttcaccttcagcagttatgccatgaactgggtgcgacaggcgcccggcaaggggctggagtgggtcgctgctattgatgatgatggtagttacacaggctacgggtcggcggtgaagggccgtgccaccatctcgagggacaacgggcagagcacagtgaggctgcagctgaacaacctcagggctgaggacaccgccatctactactgcgccaaagctgctggtagtggttactgttatcgtggtgctaatagtagttatacttgtggtacttataacgctggtgacatcgacgcatggggccacgggaccgaagtcatcgtctcctccactagtggccaggccggccagatggactacaaagacgatgacgacaagtagtag